European Patent Application EP 4 534 559 A1, published April 9, 2025. Title: ANTI-CD40 ANTIBODY, ANTI-PD-L1×CD40 BISPECIFIC ANTIBODY, AND USE THEREOF. Applicant: FutureGen Biopharmaceutical (Beijing) Co., Ltd. Application EP. The sequence listing filed with the application follows.

SEQUENCE LISTING (96 sequences)

SEQ ID NO: 1 - protein, 11 aa, synthetic construct
  VARIANT 5: note = X1=D, G, S or T
  VARIANT 7: note = X2=R or S
  VARIANT 8: note = X3=N or S
  VARIANT 11: note = X4=N or A
RASQXIXXYLX

SEQ ID NO: 2 - skipped

SEQ ID NO: 3 - protein, 8 aa, synthetic construct
  VARIANT 4: note = X10= K , I, N , Q or S
  VARIANT 5: note = X11= S , A, N or T
  VARIANT 6: note = X12 =L , Y or F
QQGXXXPW

SEQ ID NO: 4 - protein, 6 aa, synthetic construct
  VARIANT 2: note = X13 =N or D
SXYYMS

SEQ ID NO: 5 - protein, 10 aa, synthetic construct
  VARIANT 8: note = X14= A or G
FIRNKANXYT

SEQ ID NO: 6 - protein, 12 aa, synthetic construct
  VARIANT 4: note = X15= L or I
  VARIANT 5: note = X16= K or R
  VARIANT 6: note = X17= V, K , I or Q
  VARIANT 12: note = X18= L or V
YGGXXXGWYFDX

SEQ ID NO: 7 - protein, 11 aa, synthetic construct
RASQDIRNYLN

SEQ ID NO: 8 - protein, 11 aa, synthetic construct
RASQGIRNYLN

SEQ ID NO: 9 - protein, 11 aa, synthetic construct
RASQSISNYLA

SEQ ID NO: 10 - protein, 11 aa, synthetic construct
RASQTISSYLN

SEQ ID NO: 11 - protein, 7 aa, synthetic construct
YTSRLQS

SEQ ID NO: 12 - protein, 7 aa, synthetic construct
YTSRRDS

SEQ ID NO: 13 - protein, 7 aa, synthetic construct
YTSSLQS

SEQ ID NO: 14 - protein, 7 aa, synthetic construct
AASSLQS

SEQ ID NO: 15 - protein, 7 aa, synthetic construct
YTSTLQS

SEQ ID NO: 16 - protein, 8 aa, synthetic construct
QQGQSFPW

SEQ ID NO: 17 - protein, 8 aa, synthetic construct
QQGKTLPW

SEQ ID NO: 18 - protein, 8 aa, synthetic construct
QQGINLPW

SEQ ID NO: 19 - protein, 8 aa, synthetic construct
QQGSSYPW

SEQ ID NO: 20 - protein, 8 aa, synthetic construct
QQGNAYPW

SEQ ID NO: 21 - protein, 6 aa, synthetic construct
SNYYMS

SEQ ID NO: 22 - protein, 6 aa, synthetic construct
SDYYMS

SEQ ID NO: 23 - protein, 10 aa, synthetic construct
FIRNKANAYT

SEQ ID NO: 24 - protein, 10 aa, synthetic construct
FIRNKANGYT

SEQ ID NO: 25 - protein, 12 aa, synthetic construct
YGGIRVGWYFDL

SEQ ID NO: 26 - protein, 12 aa, synthetic construct
YGGLRQGWYFDV

SEQ ID NO: 27 - protein, 12 aa, synthetic construct
YGGLKKGWYFDL

SEQ ID NO: 28 - protein, 12 aa, synthetic construct
YGGLKVGWYFDL

SEQ ID NO: 29 - protein, 12 aa, synthetic construct
YGGLKIGWYFDL

SEQ ID NO: 30 - protein, 107 aa, synthetic construct
DIQMTQSPSSLSASVGDRVTITCRASQDIRNYLNWYQQKPGKAPKLLIYYTSRLQSGVPSRFSGSGSGTDYTLTISSLQPEDFATYYCQQGQSFPWTFGGGTKVEIK

SEQ ID NO: 31 - protein, 123 aa, synthetic construct
EVQLVESGGGLVQPGGSLRLSCAASGFTFSNYYMSWVRQAPGKGLEWVAFIRNKANAYTTEYAASVKGRFTISRDNSKSTLYLQMNSLRAEDTAVYYCARYGGIRVGWYFDLWGQGTLVTVSS

SEQ ID NO: 32 - protein, 107 aa, synthetic construct
DIQMTQSPSSLSASVGDRVTITCRASQDIRNYLNWYQQKPGKAPKLLIYYTSRRDSGVPSRFSGSGSGTDYTLTISSLQPEDFATYFCQQGKTLPWTFGGGTKVEIK

SEQ ID NO: 33 - protein, 123 aa, synthetic construct
EVQLVESGGGLVQPGGSLRLSCAASGFTFSDYYMSWVRQAPGKGLEWVGFIRNKANGYTTEYAASVKGRFTISRDNSKNTLYLQMNSLRAEDTAVYYCARYGGLRQGWYFDVWGQGTLVTVSS

SEQ ID NO: 34 - protein, 123 aa, synthetic construct
EVQLVESGGGLVQPGGSLRLSCAASGFTFSDYYMSWVRQAPGKGLEWVGFIRNKANAYTTEYAASVKGRFTISRDNSKNTLYLQMNSLRAEDTAVYYCARYGGLRQGWYFDVWGQGTLVTVSS

SEQ ID NO: 35 - protein, 107 aa, synthetic construct
DIQMTQSPSSLSASVGDRVTITCRASQGIRNYLNWYQQKPGKAPKLLIYYTSSLQSGVPSRFSGSGSGTDYTLTISSLQPEDFATYYCQQGINLPWTFGGGTKVEIK

SEQ ID NO: 36 - protein, 123 aa, synthetic construct
EVQLVESGGGLVQPGGSLRLSCAASGFTFSDYYMSWVRQAPGKGLEWVGFIRNKANGYTTEYAASVKGRFTISRDNSKSTLYLQMNSLRAEDTAVYYCARYGGLKKGWYFDLWGQGTLVTVSS

SEQ ID NO: 37 - protein, 123 aa, synthetic construct
EVQLVESGGGLVQPGGSLRLSCAASGFTFSDYYMSWVRQAPGKGLEWVGFIRNKANAYTTEYAASVKGRFTISRDNSKSTLYLQMNSLRAEDTAVYYCARYGGLKKGWYFDLWGQGTLVTVSS

SEQ ID NO: 38 - protein, 107 aa, synthetic construct
DIQMTQSPSSLSASVGDRVTITCRASQSISNYLAWYQQKPGKAPKLLIYAASSLQSGVPSRFSGSGSGTDYTLTISSLQPEDFATYYCQQGSSYPWTFGGGTKVEIK

SEQ ID NO: 39 - protein, 123 aa, synthetic construct
EVQLVESGGGLVQPGGSLRLSCAASGFTFSNYYMSWVRQAPGKGLEWVGFIRNKANGYTTEYAASVKGRFTISRDNSKSTLYLQMNRLRAEDTAVYYCARYGGLKVGWYFDLWGQGTLVTVSS

SEQ ID NO: 40 - protein, 123 aa, synthetic construct
EVQLVESGGGLVQPGGSLRLSCAASGFTFSNYYMSWVRQAPGKGLEWVGFIRNKANAYTTEYAASVKGRFTISRDNSKSTLYLQMNRLRAEDTAVYYCARYGGLKVGWYFDLWGQGTLVTVSS

SEQ ID NO: 41 - protein, 107 aa, synthetic construct
DIQMTQSPSSLSASVGDRVTITCRASQTISSYLNWYQQKPGKAPKLLIYYTSTLQSGVPSRFSGSGSGTDYTLTISSLQPEDFATYYCQQGNAYPWTFGGGTKVEIK

SEQ ID NO: 42 - protein, 123 aa, synthetic construct
EVQLVESGGGLVQPGGSLRLSCAASGFTFSNYYMSWVRQAPGKGLEWVGFIRNKANGYTTEYAASVKGRFTISRDNSKSTLYLQMNSLRAEDTAVYYCARYGGLKIGWYFDLWGQGTLVTVSS

SEQ ID NO: 43 - protein, 123 aa, synthetic construct
EVQLVESGGGLVQPGGSLRLSCAASGFTFSNYYMSWVRQAPGKGLEWVGFIRNKANAYTTEYAASVKGRFTISRDNSKSTLYLQMNSLRAEDTAVYYCARYGGLKIGWYFDLWGQGTLVTVSS

SEQ ID NO: 44 - protein, 107 aa, synthetic construct [sequence omitted]

SEQ ID NO: 45 - protein, 325 aa, synthetic construct
ASTKGPSVFPLAPCSRSTSESTAALGCLVKDYFPEPVTVSWNSGALTSGVHTFPAVLQSSGLYSLSSVVTVPSSNFGTQTYTCNVDHKPSNTKVDKTVERKCCVECPPCPAPPVAGPSVFLFPPKPKDTLMISRTPEVTCVVVDVSHEDPEVQFNWYVDGVEVHNAKTKPREEQFNSTFRVVSVLTVVHQDWLNGKEYKCKVSNKGLPAPIEKTISKTKGQPREPQVYTLPPSREEMTKNQVSLTCLVKGFYPSDIAVEWESNGQPENNYKTTPPMLDSDGSFFLYSKLTVDKSRWQQGNVFSCSVMHEALHNHYTQKSLSLSPG

SEQ ID NO: 46 - protein, 6 aa, synthetic construct
DYYTQC

SEQ ID NO: 47 - protein, 10 aa, synthetic construct
CISSSEGSTY

SEQ ID NO: 48 - protein, 14 aa, synthetic construct
RKGGPLTIENFFDY

SEQ ID NO: 49 - protein, 123 aa, synthetic construct
EVQLVESGGGLVQPGGSLRLSCAASGFTFDYYTQCWFRQAPGKEREWVSCISSSEGSTYYADSVKGRFTISRDNSKNTVYLQMNSLKTEDTAVYYCAARKGGPLTIENFFDYWGQGTQVTVSS

SEQ ID NO: 50 - protein, 214 aa, synthetic construct
DIQMTQSPSSLSASVGDRVTITCRASQDIRNYLNWYQQKPGKAPKLLIYYTSRLQSGVPSRFSGSGSGTDYTLTISSLQPEDFATYYCQQGQSFPWTFGGGTKVEIKRTVAAPSVFIFPPSDEQLKSGTASVVCLLNNFYPREAKVQWKVDNALQSGNSQESVTEQDSKDSTYSLSSTLTLSKADYEKHKVYACEVTHQGLSSPVTKSFNRGEC

SEQ ID NO: 51 - protein, 587 aa, synthetic construct
EVQLVESGGGLVQPGGSLRLSCAASGFTFSNYYMSWVRQAPGKGLEWVAFIRNKANAYTTEYAASVKGRFTISRDNSKSTLYLQMNSLRAEDTAVYYCARYGGIRVGWYFDLWGQGTLVTVSSASTKGPSVFPLAPCSRSTSESTAALGCLVKDYFPEPVTVSWNSGALTSGVHTFPAVLQSSGLYSLSSVVTVPSSNFGTQTYTCNVDHKPSNTKVDKTVERKCCVECPPCPAPPVAGPSVFLFPPKPKDTLMISRTPEVTCVVVDVSHEDPEVQFNWYVDGVEVHNAKTKPREEQFNSTFRVVSVLTVVHQDWLNGKEYKCKVSNKGLPAPIEKTISKTKGQPREPQVYTLPPSREEMTKNQVSLTCLVKGFYPSDIAVEWESNGQPENNYKTTPPMLDSDGSFFLYSKLTVDKSRWQQGNVFSCSVMHEALHNHYTQKSLSLSPGGGGGSGGGGSGGGGSGEVQLVESGGGLVQPGGSLRLSCAASGFTFDYYTQCWFRQAPGKEREWVSCISSSEGSTYYADSVKGRFTISRDNSKNTVYLQMNSLKTEDTAVYYCAARKGGPLTIENFFDYWGQGTQVTVSS

SEQ ID NO: 52 - protein, 214 aa, synthetic construct
DIQMTQSPSSLSASVGDRVTITCRASQDIRNYLNWYQQKPGKAPKLLIYYTSRRDSGVPSRFSGSGSGTDYTLTISSLQPEDFATYFCQQGKTLPWTFGGGTKVEIKRTVAAPSVFIFPPSDEQLKSGTASVVCLLNNFYPREAKVQWKVDNALQSGNSQESVTEQDSKDSTYSLSSTLTLSKADYEKHKVYACEVTHQGLSSPVTKSFNRGEC

SEQ ID NO: 53 - protein, 587 aa, synthetic construct
EVQLVESGGGLVQPGGSLRLSCAASGFTFSDYYMSWVRQAPGKGLEWVGFIRNKANGYTTEYAASVKGRFTISRDNSKNTLYLQMNSLRAEDTAVYYCARYGGLRQGWYFDVWGQGTLVTVSSASTKGPSVFPLAPCSRSTSESTAALGCLVKDYFPEPVTVSWNSGALTSGVHTFPAVLQSSGLYSLSSVVTVPSSNFGTQTYTCNVDHKPSNTKVDKTVERKCCVECPPCPAPPVAGPSVFLFPPKPKDTLMISRTPEVTCVVVDVSHEDPEVQFNWYVDGVEVHNAKTKPREEQFNSTFRVVSVLTVVHQDWLNGKEYKCKVSNKGLPAPIEKTISKTKGQPREPQVYTLPPSREEMTKNQVSLTCLVKGFYPSDIAVEWESNGQPENNYKTTPPMLDSDGSFFLYSKLTVDKSRWQQGNVFSCSVMHEALHNHYTQKSLSLSPGGGGGSGGGGSGGGGSGEVQLVESGGGLVQPGGSLRLSCAASGFTFDYYTQCWFRQAPGKEREWVSCISSSEGSTYYADSVKGRFTISRDNSKNTVYLQMNSLKTEDTAVYYCAARKGGPLTIENFFDYWGQGTQVTVSS

SEQ ID NO: 54 - protein, 214 aa, synthetic construct
DIQMTQSPSSLSASVGDRVTITCRASQGIRNYLNWYQQKPGKAPKLLIYYTSSLQSGVPSRFSGSGSGTDYTLTISSLQPEDFATYYCQQGINLPWTFGGGTKVEIKRTVAAPSVFIFPPSDEQLKSGTASVVCLLNNFYPREAKVQWKVDNALQSGNSQESVTEQDSKDSTYSLSSTLTLSKADYEKHKVYACEVTHQGLSSPVTKSFNRGEC

SEQ ID NO: 55 - protein, 587 aa, synthetic construct
EVQLVESGGGLVQPGGSLRLSCAASGFTFSDYYMSWVRQAPGKGLEWVGFIRNKANGYTTEYAASVKGRFTISRDNSKSTLYLQMNSLRAEDTAVYYCARYGGLKKGWYFDLWGQGTLVTVSSASTKGPSVFPLAPCSRSTSESTAALGCLVKDYFPEPVTVSWNSGALTSGVHTFPAVLQSSGLYSLSSVVTVPSSNFGTQTYTCNVDHKPSNTKVDKTVERKCCVECPPCPAPPVAGPSVFLFPPKPKDTLMISRTPEVTCVVVDVSHEDPEVQFNWYVDGVEVHNAKTKPREEQFNSTFRVVSVLTVVHQDWLNGKEYKCKVSNKGLPAPIEKTISKTKGQPREPQVYTLPPSREEMTKNQVSLTCLVKGFYPSDIAVEWESNGQPENNYKTTPPMLDSDGSFFLYSKLTVDKSRWQQGNVFSCSVMHEALHNHYTQKSLSLSPGGGGGSGGGGSGGGGSGEVQLVESGGGLVQPGGSLRLSCAASGFTFDYYTQCWFRQAPGKEREWVSCISSSEGSTYYADSVKGRFTISRDNSKNTVYLQMNSLKTEDTAVYYCAARKGGPLTIENFFDYWGQGTQVTVSS

SEQ ID NO: 56 - protein, 214 aa, synthetic construct
DIQMTQSPSSLSASVGDRVTITCRASQSISNYLAWYQQKPGKAPKLLIYAASSLQSGVPSRFSGSGSGTDYTLTISSLQPEDFATYYCQQGSSYPWTFGGGTKVEIKRTVAAPSVFIFPPSDEQLKSGTASVVCLLNNFYPREAKVQWKVDNALQSGNSQESVTEQDSKDSTYSLSSTLTLSKADYEKHKVYACEVTHQGLSSPVTKSFNRGEC

SEQ ID NO: 57 - protein, 587 aa, synthetic construct
EVQLVESGGGLVQPGGSLRLSCAASGFTFSNYYMSWVRQAPGKGLEWVGFIRNKANGYTTEYAASVKGRFTISRDNSKSTLYLQMNRLRAEDTAVYYCARYGGLKVGWYFDLWGQGTLVTVSSASTKGPSVFPLAPCSRSTSESTAALGCLVKDYFPEPVTVSWNSGALTSGVHTFPAVLQSSGLYSLSSVVTVPSSNFGTQTYTCNVDHKPSNTKVDKTVERKCCVECPPCPAPPVAGPSVFLFPPKPKDTLMISRTPEVTCVVVDVSHEDPEVQFNWYVDGVEVHNAKTKPREEQFNSTFRVVSVLTVVHQDWLNGKEYKCKVSNKGLPAPIEKTISKTKGQPREPQVYTLPPSREEMTKNQVSLTCLVKGFYPSDIAVEWESNGQPENNYKTTPPMLDSDGSFFLYSKLTVDKSRWQQGNVFSCSVMHEALHNHYTQKSLSLSPGGGGGSGGGGSGGGGSGEVQLVESGGGLVQPGGSLRLSCAASGFTFDYYTQCWFRQAPGKEREWVSCISSSEGSTYYADSVKGRFTISRDNSKNTVYLQMNSLKTEDTAVYYCAARKGGPLTIENFFDYWGQGTQVTVSS

SEQ ID NO: 58 - protein, 214 aa, synthetic construct
DIQMTQSPSSLSASVGDRVTITCRASQTISSYLNWYQQKPGKAPKLLIYYTSTLQSGVPSRFSGSGSGTDYTLTISSLQPEDFATYYCQQGNAYPWTFGGGTKVEIKRTVAAPSVFIFPPSDEQLKSGTASVVCLLNNFYPREAKVQWKVDNALQSGNSQESVTEQDSKDSTYSLSSTLTLSKADYEKHKVYACEVTHQGLSSPVTKSFNRGEC

SEQ ID NO: 59 - protein, 587 aa, synthetic construct
EVQLVESGGGLVQPGGSLRLSCAASGFTFSNYYMSWVRQAPGKGLEWVGFIRNKANGYTTEYAASVKGRFTISRDNSKSTLYLQMNSLRAEDTAVYYCARYGGLKIGWYFDLWGQGTLVTVSSASTKGPSVFPLAPCSRSTSESTAALGCLVKDYFPEPVTVSWNSGALTSGVHTFPAVLQSSGLYSLSSVVTVPSSNFGTQTYTCNVDHKPSNTKVDKTVERKCCVECPPCPAPPVAGPSVFLFPPKPKDTLMISRTPEVTCVVVDVSHEDPEVQFNWYVDGVEVHNAKTKPREEQFNSTFRVVSVLTVVHQDWLNGKEYKCKVSNKGLPAPIEKTISKTKGQPREPQVYTLPPSREEMTKNQVSLTCLVKGFYPSDIAVEWESNGQPENNYKTTPPMLDSDGSFFLYSKLTVDKSRWQQGNVFSCSVMHEALHNHYTQKSLSLSPGGGGGSGGGGSGGGGSGEVQLVESGGGLVQPGGSLRLSCAASGFTFDYYTQCWFRQAPGKEREWVSCISSSEGSTYYADSVKGRFTISRDNSKNTVYLQMNSLKTEDTAVYYCAARKGGPLTIENFFDYWGQGTQVTVSS

SEQ ID NO: 60 - protein, 587 aa, synthetic construct
EVQLVESGGGLVQPGGSLRLSCAASGFTFSDYYMSWVRQAPGKGLEWVGFIRNKANAYTTEYAASVKGRFTISRDNSKNTLYLQMNSLRAEDTAVYYCARYGGLRQGWYFDVWGQGTLVTVSSASTKGPSVFPLAPCSRSTSESTAALGCLVKDYFPEPVTVSWNSGALTSGVHTFPAVLQSSGLYSLSSVVTVPSSNFGTQTYTCNVDHKPSNTKVDKTVERKCCVECPPCPAPPVAGPSVFLFPPKPKDTLMISRTPEVTCVVVDVSHEDPEVQFNWYVDGVEVHNAKTKPREEQFNSTFRVVSVLTVVHQDWLNGKEYKCKVSNKGLPAPIEKTISKTKGQPREPQVYTLPPSREEMTKNQVSLTCLVKGFYPSDIAVEWESNGQPENNYKTTPPMLDSDGSFFLYSKLTVDKSRWQQGNVFSCSVMHEALHNHYTQKSLSLSPGGGGGSGGGGSGGGGSGEVQLVESGGGLVQPGGSLRLSCAASGFTFDYYTQCWFRQAPGKEREWVSCISSSEGSTYYADSVKGRFTISRDNSKNTVYLQMNSLKTEDTAVYYCAARKGGPLTIENFFDYWGQGTQVTVSS

SEQ ID NO: 61 - protein, 587 aa, synthetic construct
EVQLVESGGGLVQPGGSLRLSCAASGFTFSDYYMSWVRQAPGKGLEWVGFIRNKANAYTTEYAASVKGRFTISRDNSKSTLYLQMNSLRAEDTAVYYCARYGGLKKGWYFDLWGQGTLVTVSSASTKGPSVFPLAPCSRSTSESTAALGCLVKDYFPEPVTVSWNSGALTSGVHTFPAVLQSSGLYSLSSVVTVPSSNFGTQTYTCNVDHKPSNTKVDKTVERKCCVECPPCPAPPVAGPSVFLFPPKPKDTLMISRTPEVTCVVVDVSHEDPEVQFNWYVDGVEVHNAKTKPREEQFNSTFRVVSVLTVVHQDWLNGKEYKCKVSNKGLPAPIEKTISKTKGQPREPQVYTLPPSREEMTKNQVSLTCLVKGFYPSDIAVEWESNGQPENNYKTTPPMLDSDGSFFLYSKLTVDKSRWQQGNVFSCSVMHEALHNHYTQKSLSLSPGGGGGSGGGGSGGGGSGEVQLVESGGGLVQPGGSLRLSCAASGFTFDYYTQCWFRQAPGKEREWVSCISSSEGSTYYADSVKGRFTISRDNSKNTVYLQMNSLKTEDTAVYYCAARKGGPLTIENFFDYWGQGTQVTVSS

SEQ ID NO: 62 - protein, 587 aa, synthetic construct
EVQLVESGGGLVQPGGSLRLSCAASGFTFSNYYMSWVRQAPGKGLEWVGFIRNKANAYTTEYAASVKGRFTISRDNSKSTLYLQMNRLRAEDTAVYYCARYGGLKVGWYFDLWGQGTLVTVSSASTKGPSVFPLAPCSRSTSESTAALGCLVKDYFPEPVTVSWNSGALTSGVHTFPAVLQSSGLYSLSSVVTVPSSNFGTQTYTCNVDHKPSNTKVDKTVERKCCVECPPCPAPPVAGPSVFLFPPKPKDTLMISRTPEVTCVVVDVSHEDPEVQFNWYVDGVEVHNAKTKPREEQFNSTFRVVSVLTVVHQDWLNGKEYKCKVSNKGLPAPIEKTISKTKGQPREPQVYTLPPSREEMTKNQVSLTCLVKGFYPSDIAVEWESNGQPENNYKTTPPMLDSDGSFFLYSKLTVDKSRWQQGNVFSCSVMHEALHNHYTQKSLSLSPGGGGGSGGGGSGGGGSGEVQLVESGGGLVQPGGSLRLSCAASGFTFDYYTQCWFRQAPGKEREWVSCISSSEGSTYYADSVKGRFTISRDNSKNTVYLQMNSLKTEDTAVYYCAARKGGPLTIENFFDYWGQGTQVTVSS

SEQ ID NO: 63 - protein, 587 aa, synthetic construct
EVQLVESGGGLVQPGGSLRLSCAASGFTFSNYYMSWVRQAPGKGLEWVGFIRNKANAYTTEYAASVKGRFTISRDNSKSTLYLQMNSLRAEDTAVYYCARYGGLKIGWYFDLWGQGTLVTVSSASTKGPSVFPLAPCSRSTSESTAALGCLVKDYFPEPVTVSWNSGALTSGVHTFPAVLQSSGLYSLSSVVTVPSSNFGTQTYTCNVDHKPSNTKVDKTVERKCCVECPPCPAPPVAGPSVFLFPPKPKDTLMISRTPEVTCVVVDVSHEDPEVQFNWYVDGVEVHNAKTKPREEQFNSTFRVVSVLTVVHQDWLNGKEYKCKVSNKGLPAPIEKTISKTKGQPREPQVYTLPPSREEMTKNQVSLTCLVKGFYPSDIAVEWESNGQPENNYKTTPPMLDSDGSFFLYSKLTVDKSRWQQGNVFSCSVMHEALHNHYTQKSLSLSPGGGGGSGGGGSGGGGSGEVQLVESGGGLVQPGGSLRLSCAASGFTFDYYTQCWFRQAPGKEREWVSCISSSEGSTYYADSVKGRFTISRDNSKNTVYLQMNSLKTEDTAVYYCAARKGGPLTIENFFDYWGQGTQVTVSS

SEQ ID NO: 64 - protein, 123 aa, synthetic construct
  VARIANT 31: note = X19=N or D
  VARIANT 49: note = X20=G or A
  VARIANT 57: note = X21=A or G
  VARIANT 79: note = X22=N or S
  VARIANT 87: note = X23=R or S
  VARIANT 104: note = X24=L or I
  VARIANT 105: note = X25=K or R
  VARIANT 106: note = X26=V, K, I or Q
  VARIANT 112: note = X27=L or V
EVQLVESGGGLVQPGGSLRLSCAASGFTFSXYYMSWVRQAPGKGLEWVXFIRNKANXYTTEYAASVKGRFTISRDNSKXTLYLQMNXLRAEDTAVYYCARYGGXXXGWYFDXWGQGTLVTVSS

SEQ ID NO: 65 - protein, 107 aa, synthetic construct
  VARIANT 28: note = X28=D, G, S or T
  VARIANT 30: note = X29=R or S
  VARIANT 31: note = X30=N or S
  VARIANT 34: note = X31=N or A
  VARIANT 50: note = X32=Y or A
  VARIANT 51: note = X33=T or A
  VARIANT 53: note = X34=S, R or T
  VARIANT 54: note = X35=L or R
  VARIANT 55: note = X36=Q or D
  VARIANT 87: note = X37=Y or F
  VARIANT 92: note = X38=K, I , N , Q or S
  VARIANT 93: note = X39=S, A, N or T
  VARIANT 94: note = X40=L , Y or F
DIQMTQSPSSLSASVGDRVTITCRASQXIXXYLXWYQQKPGKAPKLLIYXXSXXXSGVPSRFSGSGSGTDYTLTISSLQPEDFATYXCQQGXXXPWTFGGGTKVEIK

SEQ ID NO: 66 - protein, 123 aa, synthetic construct
  VARIANT 29: note = X48=L or F
  VARIANT 30: note = X41=D or E
  VARIANT 33: note = X42=S or T
  VARIANT 34: note = X43=K or Q
  VARIANT 52: note = X44=G or S
  VARIANT 53: note = X45=S or T
  VARIANT 55: note = X46=D or E
  VARIANT 75: note = X49=A or S
  VARIANT 87: note = X50=K or R
  VARIANT 88: note = X51=A or T
  VARIANT 100: note = X47=K or N
EVQLVESGGGLVQPGGSLRLSCAASGFTXXYYXXCWFRQAPGKEREWVSCIXXSXGSTYYADSVKGRFTISRDNXKNTVYLQMNSLXXEDTAVYYCAARXGGPLTIENFFDYWGQGTQVTVSS

SEQ ID NO: 67 - protein, 6 aa, synthetic construct
DYYSKC

SEQ ID NO: 68 - protein, 10 aa, synthetic construct
CIGSSDGSTY

SEQ ID NO: 69 - protein, 14 aa, synthetic construct
RNGGPLTIENFFDY

SEQ ID NO: 70 - protein, 6 aa, synthetic construct
EYYTKC

SEQ ID NO: 71 - protein, 10 aa, synthetic construct
CISTSEGSTY

SEQ ID NO: 72 - protein, 123 aa, synthetic construct
EVQLVESGGGLVQPGGSLRLSCAASGFTLDYYSKCWFRQAPGKEREWVSCIGSSDGSTYYADSVKGRFTISRDNAKNTVYLQMNSLRAEDTAVYYCAARNGGPLTIENFFDYWGQGTQVTVSS

SEQ ID NO: 73 - protein, 123 aa, synthetic construct
EVQLVESGGGLVQPGGSLRLSCAASGFTFEYYTKCWFRQAPGKEREWVSCISTSEGSTYYADSVKGRFTISRDNAKNTVYLQMNSLRAEDTAVYYCAARKGGPLTIENFFDYWGQGTQVTVSS

SEQ ID NO: 74 - protein, 123 aa, synthetic construct
EVQLVESGGGLVQPGGSLRLSCAASGFTFDYYTQCWFRQAPGKEREWVSCISSSEGSTYYADSVKGRFTISRDNAKNTVYLQMNSLRAEDTAVYYCAARKGGPLTIENFFDYWGQGTQVTVSS

SEQ ID NO: 75 - skipped

SEQ ID NO: 76 - protein, 10 aa, synthetic construct
  VARIANT 3: note = X44=G or S
  VARIANT 4: note = X45=S or T
  VARIANT 6: note = X46=D or E
CIXXSXGSTY

SEQ ID NO: 77 - protein, 14 aa, synthetic construct
  VARIANT 2: note = X47=K or N
RXGGPLTIENFFDY

SEQ ID NO: 78 - protein, 29 aa, synthetic construct
EVQLVESGGGLVQPGGSLRLSCAASGFTL

SEQ ID NO: 79 - protein, 14 aa, synthetic construct
WFRQAPGKEREWVS

SEQ ID NO: 80 - protein, 38 aa, synthetic construct
ADSVKGRFTISRDNAKNTVYLQMNSLRAEDTAVYYCAA

SEQ ID NO: 81 - protein, 214 aa, synthetic construct; identical to SEQ ID NO: 52

SEQ ID NO: 82 - protein, 29 aa, synthetic construct
EVQLVESGGGLVQPGGSLRLSCAASGFTF

SEQ ID NO: 83 - protein, 39 aa, synthetic construct
YADSVKGRFTISRDNSKNTVYLQMNSLKTEDTAVYYCAA

SEQ ID NO: 84 - protein, 11 aa, synthetic construct
WGQGTQVTVSS

SEQ ID NO: 85 - protein, 29 aa, synthetic construct
  VARIANT 29: note = X48=L or F
EVQLVESGGGLVQPGGSLRLSCAASGFTX

SEQ ID NO: 86 - protein, 39 aa, synthetic construct
  VARIANT 16: note = X49=A or S
  VARIANT 28: note = X50=K or R
  VARIANT 29: note = X51= A or T
YADSVKGRFTISRDNXKNTVYLQMNSLXXEDTAVYYCAA

SEQ ID NO: 87 - protein, 448 aa, synthetic construct
EVQLVESGGGLVQPGGSLRLSCAASGFTFSDYYMSWVRQAPGKGLEWVGFIRNKANAYTTEYAASVKGRFTISRDNSKNTLYLQMNSLRAEDTAVYYCARYGGLRQGWYFDVWGQGTLVTVSSASTKGPSVFPLAPCSRSTSESTAALGCLVKDYFPEPVTVSWNSGALTSGVHTFPAVLQSSGLYSLSSVVTVPSSNFGTQTYTCNVDHKPSNTKVDKTVERKCCVECPPCPAPPVAGPSVFLFPPKPKDTLMISRTPEVTCVVVDVSHEDPEVQFNWYVDGVEVHNAKTKPREEQFNSTFRVVSVLTVVHQDWLNGKEYKCKVSNKGLPAPIEKTISKTKGQPREPQVYTLPPSREEMTKNQVSLTCLVKGFYPSDIAVEWESNGQPENNYKTTPPMLDSDGSFFLYSKLTVDKSRWQQGNVFSCSVMHEALHNHYTQKSLSLSPG

SEQ ID NO: 88 - protein, 231 aa, synthetic construct
EPKSCDKTHTCPPCPAPELLGGPSVFLFPPKPKDTLMISRTPEVTCVVVDVSHEDPEVKFNWYVDGVEVHNAKTKPREEQYNSTYRVVSVLTVLHQDWLNGKEYKCKVSNKALPAPIEKTISKAKGQPREPQVYTLPPSREEMTKNQVSLTCLVKGFYPSDIAVEWESNGQPENNYKTTPPVLDSDGSFFLYSKLTVDKSRWQQGNVFSCSVMHEALHNHYTQKSLSLSPG

SEQ ID NO: 89 - protein, 16 aa, synthetic construct
GGGGSGGGGSGGGGSG

SEQ ID NO: 90 - protein, 370 aa, synthetic construct
EVQLVESGGGLVQPGGSLRLSCAASGFTLDYYSKCWFRQAPGKEREWVSCIGSSDGSTYYADSVKGRFTISRDNAKNTVYLQMNSLRAEDTAVYYCAARNGGPLTIENFFDYWGQGTQVTVSSGGGGSGGGGSGGGGSGEPKSCDKTHTCPPCPAPELLGGPSVFLFPPKPKDTLMISRTPEVTCVVVDVSHEDPEVKFNWYVDGVEVHNAKTKPREEQYNSTYRVVSVLTVLHQDWLNGKEYKCKVSNKALPAPIEKTISKAKGQPREPQVYTLPPSREEMTKNQVSLTCLVKGFYPSDIAVEWESNGQPENNYKTTPPVLDSDGSFFLYSKLTVDKSRWQQGNVFSCSVMHEALHNHYTQKSLSLSPG

SEQ ID NO: 91 - protein, 370 aa, synthetic construct
EVQLVESGGGLVQPGGSLRLSCAASGFTFEYYTKCWFRQAPGKEREWVSCISTSEGSTYYADSVKGRFTISRDNAKNTVYLQMNSLRAEDTAVYYCAARKGGPLTIENFFDYWGQGTQVTVSSGGGGSGGGGSGGGGSGEPKSCDKTHTCPPCPAPELLGGPSVFLFPPKPKDTLMISRTPEVTCVVVDVSHEDPEVKFNWYVDGVEVHNAKTKPREEQYNSTYRVVSVLTVLHQDWLNGKEYKCKVSNKALPAPIEKTISKAKGQPREPQVYTLPPSREEMTKNQVSLTCLVKGFYPSDIAVEWESNGQPENNYKTTPPVLDSDGSFFLYSKLTVDKSRWQQGNVFSCSVMHEALHNHYTQKSLSLSPG

SEQ ID NO: 92 - protein, 370 aa, synthetic construct
EVQLVESGGGLVQPGGSLRLSCAASGFTFDYYTQCWFRQAPGKEREWVSCISSSEGSTYYADSVKGRFTISRDNAKNTVYLQMNSLRAEDTAVYYCAARKGGPLTIENFFDYWGQGTQVTVSSGGGGSGGGGSGGGGSGEPKSCDKTHTCPPCPAPELLGGPSVFLFPPKPKDTLMISRTPEVTCVVVDVSHEDPEVKFNWYVDGVEVHNAKTKPREEQYNSTYRVVSVLTVLHQDWLNGKEYKCKVSNKALPAPIEKTISKAKGQPREPQVYTLPPSREEMTKNQVSLTCLVKGFYPSDIAVEWESNGQPENNYKTTPPVLDSDGSFFLYSKLTVDKSRWQQGNVFSCSVMHEALHNHYTQKSLSLSPG

SEQ ID NO: 93 - protein, 370 aa, synthetic construct
EVQLVESGGGLVQPGGSLRLSCAASGFTFDYYTQCWFRQAPGKEREWVSCISSSEGSTYYADSVKGRFTISRDNSKNTVYLQMNSLKTEDTAVYYCAARKGGPLTIENFFDYWGQGTQVTVSSGGGGSGGGGSGGGGSGEPKSCDKTHTCPPCPAPELLGGPSVFLFPPKPKDTLMISRTPEVTCVVVDVSHEDPEVKFNWYVDGVEVHNAKTKPREEQYNSTYRVVSVLTVLHQDWLNGKEYKCKVSNKALPAPIEKTISKAKGQPREPQVYTLPPSREEMTKNQVSLTCLVKGFYPSDIAVEWESNGQPENNYKTTPPVLDSDGSFFLYSKLTVDKSRWQQGNVFSCSVMHEALHNHYTQKSLSLSPG

SEQ ID NO: 94 - protein, 448 aa, synthetic construct
EVQLVESGGGLVQPGGSLRLSCAASGFTFSNYYMSWVRQAPGKGLEWVGFIRNKANAYTTEYAASVKGRFTISRDNSKSTLYLQMNRLRAEDTAVYYCARYGGLKVGWYFDLWGQGTLVTVSSASTKGPSVFPLAPCSRSTSESTAALGCLVKDYFPEPVTVSWNSGALTSGVHTFPAVLQSSGLYSLSSVVTVPSSNFGTQTYTCNVDHKPSNTKVDKTVERKCCVECPPCPAPPVAGPSVFLFPPKPKDTLMISRTPEVTCVVVDVSHEDPEVQFNWYVDGVEVHNAKTKPREEQFNSTFRVVSVLTVVHQDWLNGKEYKCKVSNKGLPAPIEKTISKTKGQPREPQVYTLPPSREEMTKNQVSLTCLVKGFYPSDIAVEWESNGQPENNYKTTPPMLDSDGSFFLYSKLTVDKSRWQQGNVFSCSVMHEALHNHYTQKSLSLSPG

SEQ ID NO: 95 - protein, 214 aa, synthetic construct; identical to SEQ ID NO: 56

SEQ ID NO: 96 - protein, 448 aa, synthetic construct
EVQLVESGGGLVQPGGSLRLSCAASGFTFSDYYMSWVRQAPGKGLEWVGFIRNKANGYTTEYAASVKGRFTISRDNSKNTLYLQMNSLRAEDTAVYYCARYGGLRQGWYFDVWGQGTLVTVSSASTKGPSVFPLAPCSRSTSESTAALGCLVKDYFPEPVTVSWNSGALTSGVHTFPAVLQSSGLYSLSSVVTVPSSNFGTQTYTCNVDHKPSNTKVDKTVERKCCVECPPCPAPPVAGPSVFLFPPKPKDTLMISRTPEVTCVVVDVSHEDPEVQFNWYVDGVEVHNAKTKPREEQFNSTFRVVSVLTVVHQDWLNGKEYKCKVSNKGLPAPIEKTISKTKGQPREPQVYTLPPSREEMTKNQVSLTCLVKGFYPSDIAVEWESNGQPENNYKTTPPMLDSDGSFFLYSKLTVDKSRWQQGNVFSCSVMHEALHNHYTQKSLSLSPG